European Patent Application EP 4 711 382 A1, published March 18, 2026. Title: 一种微肽MIAC的应用. Applicant: 南京安吉生物科技有限公司. Application WO. The sequence listing filed with the application follows.

SEQUENCE LISTING (4 sequences)

SEQ ID NO: 1 - protein, 51 aa, Homo sapiens
MERAGVPGFSPRRSSVEAKMQSTSCSVRKSSTVTAWPAVVLLLSWGQRRGG

SEQ ID NO: 2 - DNA, 156 bp, synthetic construct
  source 1..156: mol_type = other DNA
atggagagagcaggggtgcccgggttctctccgcggcgctcatcggtggaggcgaagatgcagagcaccagctgcagtgtcaggaagagctccacagtcaccgcctggccagccgtcgtgctgttgctgagctggggacagagaagaggcggatga

SEQ ID NO: 3 - DNA, 22 bp, synthetic construct
  source 1..22: mol_type = other DNA
atggagagagcaggggtgcccg

SEQ ID NO: 4 - DNA, 23 bp, synthetic construct
  source 1..23: mol_type = other DNA
cgcctcttctctgtccccagctc